European Patent Specification EP 3 919 628 B1, published May 14, 2025. Title: A METHOD OF DETECTING RNA. Applicant: Xenohelix. Co., Ltd. The sequence listing filed with the application follows.

SEQUENCE LISTING (25 sequences)

SEQ ID NO: 1 - DNA, 22 bp, Artificial Sequence
  Hs-RNaseP sensor DNA
aagggagtgctgacagagactg

SEQ ID NO: 2 - DNA, 24 bp, Artificial Sequence
  Hs-U6 sensor DNA
atatggaacgcttcacgaatttgc

SEQ ID NO: 3 - DNA, 20 bp, Artificial Sequence
  COVID-19 ORF7 sensor DNA
tacgccgtcaggacaagcaa

SEQ ID NO: 4 - DNA, 20 bp, Artificial Sequence
  COVID-19 N gene sensor DNA
tgcgcgacattccgaagaac

SEQ ID NO: 5 - DNA, 20 bp, Artificial Sequence
  COVID-19 RdRp gene sensor DNA
atttgttcgcgtggtttgcc

SEQ ID NO: 6 - DNA, 10 bp, Artificial Sequence
  complementary sequence of Hs-RNaseP barcode region
ttgtcttcca

SEQ ID NO: 7 - DNA, 10 bp, Artificial Sequence
  complementary sequence of Hs-RNaseP barcode region
tggaagacaa

SEQ ID NO: 8 - DNA, 10 bp, Artificial Sequence
  complementary sequence of Hs-U6 barcode region
tactaaaatt

SEQ ID NO: 9 - DNA, 10 bp, Artificial Sequence
  complementary sequence of Hs-U6 barcode region
aattttagta

SEQ ID NO: 10 - DNA, 10 bp, Artificial Sequence
  complementary sequence of COVID-19 ORF7 barcode region
attcaccatt

SEQ ID NO: 11 - DNA, 10 bp, Artificial Sequence
  complementary sequence of COVID-19 ORF7 barcode region
aatggtgaat

SEQ ID NO: 12 - DNA, 10 bp, Artificial Sequence
  complementary sequence of COVID-19 N gene barcode region
ccagaacaaa

SEQ ID NO: 13 - DNA, 10 bp, Artificial Sequence
  complementary sequence of COVID-19 N gene barcode region
tttgttctgg

SEQ ID NO: 14 - DNA, 10 bp, Artificial Sequence
  complementary sequence of COVID-19 RdRp gene barcode region
tggtggacag

SEQ ID NO: 15 - DNA, 10 bp, Artificial Sequence
  complementary sequence of COVID-19 RdRp gene barcode region
ctgtccacca

SEQ ID NO: 16 - DNA, 23 bp, Artificial Sequence
  Hs_RNaseP Forward primer
cggccatcagaaggagatgaaga

SEQ ID NO: 17 - DNA, 22 bp, Artificial Sequence
  Hs_RNaseP Reverse primer
aagggagtgctgacagagactg

SEQ ID NO: 18 - DNA, 21 bp, Artificial Sequence
  Hs_U6  Forward primer
tgctcgcttcggcagcacata

SEQ ID NO: 19 - DNA, 24 bp, Artificial Sequence
  Hs_U6  Reverse primer
atatggaacgcttcacgaatttgc

SEQ ID NO: 20 - DNA, 22 bp, Artificial Sequence
  COVID-19 ORF7 Forward primer
tcttctggaacatacgagggca

SEQ ID NO: 21 - DNA, 20 bp, Artificial Sequence
  COVID-19 ORF7 Reverse primer
tacgccgtcaggacaagcaa

SEQ ID NO: 22 - DNA, 20 bp, Artificial Sequence
  COVID-19 N gene Forward primer
aagctttcggcagacgtggt

SEQ ID NO: 23 - DNA, 20 bp, Artificial Sequence
  COVID-19 N gene Reverse primer
tgcgcgacattccgaagaac

SEQ ID NO: 24 - DNA, 20 bp, Artificial Sequence
  COVID-19 RdRp gene Forward primer
agctcatgggacacttcgca

SEQ ID NO: 25 - DNA, 20 bp, Artificial Sequence
  COVID-19 RdRp gene Reverse primer
atttgttcgcgtggtttgcc